European Patent Application EP 4 438 053 A2, published October 2, 2024. Title: AN ANAPLASTIC LYMPHOMA KINASE (ALK) CANCER VACCINE AND METHODS OF USE. Applicant: CHILDREN'S MEDICAL CENTER CORPORATION. The sequence listing filed with the application follows.

SEQUENCE LISTING (89 sequences)

SEQ ID NO: 1 - protein, 9 aa, Homo sapiens
AMLDLLHVA

SEQ ID NO: 2 - protein, 10 aa, Homo sapiens
RPRPSQPSSL

SEQ ID NO: 3 - protein, 9 aa, Homo sapiens
IVRCIGVSL

SEQ ID NO: 4 - protein, 9 aa, Homo sapiens
VPRKNITLI

SEQ ID NO: 5 - protein, 9 aa, Homo sapiens
TAAEVSVRV

SEQ ID NO: 6 - protein, 1626 aa, Homo sapiens
TASSGGMGAIGLLWLLPLLLSTAAVGSGMGTGQRAGSPAAGPPLQPREPLSYSRLQRKSLAVDFVVPSLFRVYARDLLLPPSSSELKAGRPEARGSLALDCAPLLRLLGPAPGVSWTAGSPAPAEARTLSRVLKGGSVRKLRRAKQLVLELGEEAILEGCVGPPGEAAVGLLQFNLSELFSWWIRQGEGRLRIRLMPEKKASEVGREGRLSAAIRASQPRLLFQIFGTGHSSLESPTNMPSPSPDYFTWNLTWIMKDSFPFLSHRSRYGLECSFDFPCELEYSPPLHDLRNQSWSWRRIPSEEASQMDLLDGPGAERSKEMPRGSFLLLNTSADSKHTILSPWMRSSSEHCTLAVSVHRHLQPSGRYIAQLLPHNEAAREILLMPTPGKHGWTVLQGRIGRPDNPFRVALEYISSGNRSLSAVDFFALKNCSEGTSPGSKMALQSSFTCWNGTVLQLGQACDFHQDCAQGEDESQMCRKLPVGFYCNFEDGFCGWTQGTLSPHTPQWQVRTLKDARFQDHQDHALLLSTTDVPASESATVTSATFPAPIKSSPCELRMSWLIRGVLRGNVSLVLVENKTGKEQGRMVWHVAAYEGLSLWQWMVLPLLDVSDRFWLQMVAWWGQGSRAIVAFDNISISLDCYLTISGEDKILQNTAPKSRNLFERNPNKELKPGENSPRQTPIFDPTVHWLFTTCGASGPHGPTQAQCNNAYQNSNLSVEVGSEGPLKGIQIWKVPATDTYSISGYGAAGGKGGKNTMMRSHGVSVLGIFNLEKDDMLYILVGQQGEDACPSTNQLIQKVCIGENNVIEEEIRVNRSVHEWAGGGGGGGGATYVFKMKDGVPVPLIIAAGGGGRAYGAKTDTFHPERLENNSSVLGLNGNSGAAGGGGGWNDNTSLLWAGKSLQEGATGGHSCPQAMKKWGWETRGGFGGGGGGCSSGGGGGGYIGGNAASNNDPEMDGEDGVSFISPLGILYTPALKVMEGHGEVNIKHYLNCSHCEVDECHMDPESHKVICFCDHGTVLAEDGVSCIVSPTPEPHLPLSLILSVVTSALVAALVLAFSGIMIVYRRKHQELQAMQMELQSPEYKLSKLRTSTIMTDYNPNYCFAGKTSSISDLKEVPRKNITLIRGLGHGAFGEVYEGQVSGMPNDPSPLQVAVKTLPEVCSEQDELDFLMEALIISKFNHQNIVRCIGVSLQSLPRFILLELMAGGDLKSFLRETRPRPSQPSSLAMLDLLHVARDIACGCQYLEENHFIHRDIAARNCLLTCPGPGRVAKIGDFGMARDIYRASYYRKGGCAMLPVKWMPPEAFMEGIFTSKTDTWSFGVLLWEIFSLGYMPYPSKSNQEVLEFVTSGGRMDPPKNCPGPVYRIMTQCWQHQPEDRPNFAIILERIEYCTQDPDVINTALPIEYGPLVEEEEKVPVRPKDPEGVPPLLVSQQAKREEERSPAAPPPLPTTSSGKAAKKPTAAEISVRVPRGPAVEGGHVNMAFSQSNPPSELHKVHGSRNKPTSLWNPTYGSWFTEKPTKKNNPIAKKEPHDRGNLGLEGSCTVPPNVATGRLPGASLLLEPSSLTANMKEVPLFRLRHFPCGNVNYGYQQQGLPLEAATAPGAGHYEDTILKSKNSMNQPGP

SEQ ID NO: 7 - protein, 38 aa, Homo sapiens
GAAAVVAAGTSRRLCSEGRGAPRCFPAALWSATQSRGR

SEQ ID NO: 8 - protein, 1620 aa, Homo sapiens
MGAIGLLWLLPLLLSTAAVGSGMGTGQRAGSPAAGPPLQPREPLSYSRLQRKSLAVDFVVPSLFRVYARDLLLPPSSSELKAGRPEARGSLALDCAPLLRLLGPAPGVSWTAGSPAPAEARTLSRVLKGGSVRKLRRAKQLVLELGEEAILEGCVGPPGEAAVGLLQFNLSELFSWWIRQGEGRLRIRLMPEKKASEVGREGRLSAAIRASQPRLLFQIFGTGHSSLESPTNMPSPSPDYFTWNLTWIMKDSFPFLSHRSRYGLECSFDFPCELEYSPPLHDLRNQSWSWRRIPSEEASQMDLLDGPGAERSKEMPRGSFLLLNTSADSKHTILSPWMRSSSEHCTLAVSVHRHLQPSGRYIAQLLPHNEAAREILLMPTPGKHGWTVLQGRIGRPDNPFRVALEYISSGNRSLSAVDFFALKNCSEGTSPGSKMALQSSFTCWNGTVLQLGQACDFHQDCAQGEDESQMCRKLPVGFYCNFEDGFCGWTQGTLSPHTPQWQVRTLKDARFQDHQDHALLLSTTDVPASESATVTSATFPAPIKSSPCELRMSWLIRGVLRGNVSLVLVENKTGKEQGRMVWHVAAYEGLSLWQWMVLPLLDVSDRFWLQMVAWWGQGSRAIVAFDNISISLDCYLTISGEDKILQNTAPKSRNLFERNPNKELKPGENSPRQTPIFDPTVHWLFTTCGASGPHGPTQAQCNNAYQNSNLSVEVGSEGPLKGIQIWKVPATDTYSISGYGAAGGKGGKNTMMRSHGVSVLGIFNLEKDDMLYILVGQQGEDACPSTNQLIQKVCIGENNVIEEEIRVNRSVHEWAGGGGGGGGATYVFKMKDGVPVPLIIAAGGGGRAYGAKTDTFHPERLENNSSVLGLNGNSGAAGGGGGWNDNTSLLWAGKSLQEGATGGHSCPQAMKKWGWETRGGFGGGGGGCSSGGGGGGYIGGNAASNNDPEMDGEDGVSFISPLGILYTPALKVMEGHGEVNIKHYLNCSHCEVDECHMDPESHKVICFCDHGTVLAEDGVSCIVSPTPEPHLPLSLILSVVTSALVAALVLAFSGIMIVYRRKHQELQAMQMELQSPEYKLSKLRTSTIMTDYNPNYCFAGKTSSISDLKEVPRKNITLIRGLGHGAFGEVYEGQVSGMPNDPSPLQVAVKTLPEVCSEQDELDFLMEALIISKFNHQNIVRCIGVSLQSLPRFILLELMAGGDLKSFLRETRPRPSQPSSLAMLDLLHVARDIACGCQYLEENHFIHRDIAARNCLLTCPGPGRVAKIGDFGMARDIYRASYYRKGGCAMLPVKWMPPEAFMEGIFTSKTDTWSFGVLLWEIFSLGYMPYPSKSNQEVLEFVTSGGRMDPPKNCPGPVYRIMTQCWQHQPEDRPNFAIILERIEYCTQDPDVINTALPIEYGPLVEEEEKVPVRPKDPEGVPPLLVSQQAKREEERSPAAPPPLPTTSSGKAAKKPTAAEISVRVPRGPAVEGGHVNMAFSQSNPPSELHKVHGSRNKPTSLWNPTYGSWFTEKPTKKNNPIAKKEPHDRGNLGLEGSCTVPPNVATGRLPGASLLLEPSSLTANMKEVPLFRLRHFPCGNVNYGYQQQGLPLEAATAPGAGHYEDTILKSKNSMNQPGP

SEQ ID NO: 9 - DNA, 6221 bp, Homo sapiens
  source 1..6221: mol_type = unassigned DNA
ggggcggcagcggtggtagcagctggtacctcccgccgcctctgttcggagggtcgcggggcaccgaggtgctttccggccgccctctggtcggccacccaaagccgcgggcgctgatgatgggtgaggagggggcggcaagatttcgggcgcccctgccctgaacgccctcagctgctgccgccggggccgctccagtgcctgcgaactctgaggagccgaggcgccggtgagagcaaggacgctgcaaacttgcgcagcgcgggggctgggattcacgcccagaagttcagcaggcagacagtccgaagccttcccgcagcggagagatagcttgagggtgcgcaagacggcagcctccgccctcggttcccgcccagaccgggcagaagagcttggaggagccaaaaggaacgcaaaaggcggccaggacagcgtgcagcagctgggagccgccgttctcagccttaaaagttgcagagattggaggctgccccgagaggggacagaccccagctccgactgcggggggcaggagaggacggtacccaactgccacctcccttcaaccatagtagttcctctgtaccgagcgcagcgagctacagacgggggcgcggcactcggcgcggagagcgggaggctcaaggtcccagccagtgagcccagtgtgcttgagtgtctctggactcgcccctgagcttccaggtctgtttcatttagactcctgctcgcctccgtgcagttgggggaaagcaagagacttgcgcgcacgcacagtcctctggagatcaggtggaaggagccgctgggtaccaaggactgttcagagcctcttcccatctcggggagagcgaagggtgaggctgggcccggagagcagtgtaaacggcctcctccggcgggatgggagccatcgggctcctgtggctcctgccgctgctgctttccacggcagctgtgggctccgggatggggaccggccagcgcgcgggctccccagctgcggggccgccgctgcagccccgggagccactcagctactcgcgcctgcagaggaagagtctggcagttgacttcgtggtgccctcgctcttccgtgtctacgcccgggacctactgctgccaccatcctcctcggagctgaaggctggcaggcccgaggcccgcggctcgctagctctggactgcgccccgctgctcaggttgctggggccggcgccgggggtctcctggaccgccggttcaccagccccggcagaggcccggacgctgtccagggtgctgaagggcggctccgtgcgcaagctccggcgtgccaagcagttggtgctggagctgggcgaggaggcgatcttggagggttgcgtcgggccccccggggaggcggctgtggggctgctccagttcaatctcagcgagctgttcagttggtggattcgccaaggcgaagggcgactgaggatccgcctgatgcccgagaagaaggcgtcggaagtgggcagagagggaaggctgtccgcggcaattcgcgcctcccagccccgccttctcttccagatcttcgggactggtcatagctccttggaatcaccaacaaacatgccttctccttctcctgattattttacatggaatctcacctggataatgaaagactccttccctttcctgtctcatcgcagccgatatggtctggagtgcagctttgacttcccctgtgagctggagtattcccctccactgcatgacctcaggaaccagagctggtcctggcgccgcatcccctccgaggaggcctcccagatggacttgctggatgggcctggggcagagcgttctaaggagatgcccagaggctcctttctccttctcaacacctcagctgactccaagcacaccatcctgagtccgtggatgaggagcagcagtgagcactgcacactggccgtctcggtgcacaggcacctgcagccctctggaaggtacattgcccagctgctgccccacaacgaggctgcaagagagatcctcctgatgcccactccagggaagcatggttggacagtgctccagggaagaatcgggcgtccagacaacccatttcgagtggccctggaatacatctccagtggaaaccgcagcttgtctgcagtggacttctttgccctgaagaactgcagtgaaggaacatccccaggctccaagatggccctgcagagctccttcacttgttggaatgggacagtcctccagcttgggcaggcctgtgacttccaccaggactgtgcccagggagaagatgagagccagatgtgccggaaactgcctgtgggtttttactgcaactttgaagatggcttctgtggctggacccaaggcacactgtcaccccacactcctcaatggcaggtcaggaccctaaaggatgcccggttccaggaccaccaagaccatgctctattgctcagtaccactgatgtccccgcttctgaaagtgctacagtgaccagtgctacgtttcctgcaccgatcaagagctctccatgtgagctccgaatgtcctggctcattcgtggagtcttgaggggaaacgtgtccttggtgctagtggagaacaaaaccgggaaggagcaaggcaggatggtctggcatgtcgccgcctatgaaggcttgagcctgtggcagtggatggtgttgcctctcctcgatgtgtctgacaggttctggctgcagatggtcgcatggtggggacaaggatccagagccatcgtggcttttgacaatatctccatcagcctggactgctacctcaccattagcggagaggacaagatcctgcagaatacagcacccaaatcaagaaacctgtttgagagaaacccaaacaaggagctgaaacccggggaaaattcaccaagacagacccccatctttgaccctacagttcattggctgttcaccacatgtggggccagcgggccccatggccccacccaggcacagtgcaacaacgcctaccagaactccaacctgagcgtggaggtggggagcgagggccccctgaaaggcatccagatctggaaggtgccagccaccgacacctacagcatctcgggctacggagctgctggcgggaaaggcgggaagaacaccatgatgcggtcccacggcgtgtctgtgctgggcatcttcaacctggagaaggatgacatgctgtacatcctggttgggcagcagggagaggacgcctgccccagtacaaaccagttaatccagaaagtctgcattggagagaacaatgtgatagaagaagaaatccgtgtgaacagaagcgtgcatgagtgggcaggaggcggaggaggagggggtggagccacctacgtatttaagatgaaggatggagtgccggtgcccctgatcattgcagccggaggtggtggcagggcctacggggccaagacagacacgttccacccagagagactggagaataactcctcggttctagggctaaacggcaattccggagccgcaggtggtggaggtggctggaatgataacacttccttgctctgggccggaaaatctttgcaggagggtgccaccggaggacattcctgcccccaggccatgaagaagtgggggtgggagacaagagggggtttcggagggggtggaggggggtgctcctcaggtggaggaggcggaggatatataggcggcaatgcagcctcaaacaatgaccccgaaatggatggggaagatggggtttccttcatcagtccactgggcatcctgtacaccccagctttaaaagtgatggaaggccacggggaagtgaatattaagcattatctaaactgcagtcactgtgaggtagacgaatgtcacatggaccctgaaagccacaaggtcatctgcttctgtgaccacgggacggtgctggctgaggatggcgtctcctgcattgtgtcacccaccccggagccacacctgccactctcgctgatcctctctgtggtgacctctgccctcgtggccgccctggtcctggctttctccggcatcatgattgtgtaccgccggaagcaccaggagctgcaagccatgcagatggagctgcagagccctgagtacaagctgagcaagctccgcacctcgaccatcatgaccgactacaaccccaactactgctttgctggcaagacctcctccatcagtgacctgaaggaggtgccgcggaaaaacatcaccctcattcggggtctgggccatggcgcctttggggaggtgtatgaaggccaggtgtccggaatgcccaacgacccaagccccctgcaagtggctgtgaagacgctgcctgaagtgtgctctgaacaggacgaactggatttcctcatggaagccctgatcatcagcaaattcaaccaccagaacattgttcgctgcattggggtgagcctgcaatccctgccccggttcatcctgctggagctcatggcggggggagacctcaagtccttcctccgagagacccgccctcgcccgagccagccctcctccctggccatgctggaccttctgcacgtggctcgggacattgcctgtggctgtcagtatttggaggaaaaccacttcatccaccgagacattgctgccagaaactgcctcttgacctgtccaggccctggaagagtggccaagattggagacttcgggatggcccgagacatctacagggcgagctactatagaaagggaggctgtgccatgctgccagttaagtggatgcccccagaggccttcatggaaggaatattcacttctaaaacagacacatggtcctttggagtgctgctatgggaaatcttttctcttggatatatgccataccccagcaaaagcaaccaggaagttctggagtttgtcaccagtggaggccggatggacccacccaagaactgccctgggcctgtataccggataatgactcagtgctggcaacatcagcctgaagacaggcccaactttgccatcattttggagaggattgaatactgcacccaggacccggatgtaatcaacaccgctttgccgatagaatatggtccacttgtggaagaggaagagaaagtgcctgtgaggcccaaggaccctgagggggttcctcctctcctggtctctcaacaggcaaaacgggaggaggagcgcagcccagctgccccaccacctctgcctaccacctcctctggcaaggctgcaaagaaacccacagctgcagagatctctgttcgagtccctagagggccggccgtggaagggggacacgtgaatatggcattctctcagtccaaccctccttcggagttgcacaaggtccacggatccagaaacaagcccaccagcttgtggaacccaacgtacggctcctggtttacagagaaacccaccaaaaagaataatcctatagcaaagaaggagccacacgacaggggtaacctggggctggagggaagctgtactgtcccacctaacgttgcaactgggagacttccgggggcctcactgctcctagagccctcttcgctgactgccaatatgaaggaggtacctctgttcaggctacgtcacttcccttgtgggaatgtcaattacggctaccagcaacagggcttgcccttagaagccgctactgcccctggagctggtcattacgaggataccattctgaaaagcaagaatagcatgaaccagcctgggccctgagctcggtcgcacactcacttctcttccttgggatccctaagaccgtggaggagagagaggcaatggctccttcacaaaccagagaccaaatgtcacgttttgttttgtgccaacctattttgaagtaccaccaaaaaagctgtattttgaaaatgctttagaaaggttttgagcatgggttcatcctattctttcgaaagaagaaaatatcataaaaatgagtgataaatacaaggcccagatgtggttgcataaggtttttatgcatgtttgttgtatacttccttatgcttctttcaaattgtgtgtgctctgcttcaatgtagtcagaattagctgcttctatgtttcatagttggggtcatagatgtttccttgccttgttgatgtggacatgagccatttgaggggagagggaacggaaataaaggagttatttgtaatgactaaaa

SEQ ID NO: 10 - protein, 680 aa, Homo sapiens [sequence omitted]

SEQ ID NO: 11 - protein, 680 aa, Homo sapiens
MEDSMDMDMSPLRPQNYLFGCELKADKDYHFKVDNDENEHQLSLRTVSLGAGAKDELHIVEAEAMNYEGSPIKVTLATLKMSVQPTVSLGGFEITPPVVLRLKCGSGPVHISGQHLVVYRRKHQELQAMQMELQSPEYKLSKLRTSTIMTDYNPNYCFAGKTSSISDLKEVPRKNITLIRGLGHGAFGEVYEGQVSGMPNDPSPLQVAVKTLPEVCSEQDELDFLMEALIISKFNHQNIVRCIGVSLQSLPRFILLELMAGGDLKSFLRETRPRPSQPSSLAMLDLLHVARDIACGCQYLEENHFIHRDIAARNCLLTCPGPGRVAKIGDFGMARDIYRASYYRKGGCAMLPVKWMPPEAFMEGIFTSKTDTWSFGVLLWEIFSLGYMPYPSKSNQEVLEFVTSGGRMDPPKNCPGPVYRIMTQCWQHQPEDRPNFAIILERIEYCTQDPDVINTALPIEYGPLVEEEEKVPVRPKDPEGVPPLLVSQQAKREEERSPAAPPPLPTTSSGKAAKKPTAAEVSVRVPRGPAVEGGHVNMAFSQSNPPSELHKVHGSRNKPTSLWNPTYGSWFTEKPTKKNNPIAKKEPHDRGNLGLEGSCTVPPNVATGRLPGASLLLEPSSLTANMKEVPLFRLRHFPCGNVNYGYQQQGLPLEAATAPGAGHYEDTILKSKNSMNQPGP

SEQ ID NO: 12 - DNA, 2043 bp, Homo sapiens
  source 1..2043: mol_type = unassigned DNA
atggaagattcgatggacatggacatgagccccctgaggccccagaactatcttttcggttgtgaactaaaggccgacaaagattatcactttaaggtggataatgatgaaaatgagcaccagttatctttaagaacggtcagtttaggggctggtgcaaaggatgagttgcacattgttgaagcagaggcaatgaattacgaaggcagtccaattaaagtaacactggcaactttgaaaatgtctgtacagccaacggtttcccttgggggctttgaaataacaccaccagtggtcttaaggttgaagtgtggttcagggccagtgcatattagtggacagcacttagtagtgtaccgccggaagcaccaggagctgcaagccatgcagatggagctgcagagccctgagtacaagctgagcaagctccgcacctcgaccatcatgaccgactacaaccccaactactgctttgctggcaagacctcctccatcagtgacctgaaggaggtgccgcggaaaaacatcaccctcattcggggtctgggccatggcgcctttggggaggtgtatgaaggccaggtgtccggaatgcccaacgacccaagccccctgcaagtggctgtgaagacgctgcctgaagtgtgctctgaacaggacgaactggatttcctcatggaagccctgatcatcagcaaattcaaccaccagaacattgttcgctgcattggggtgagcctgcaatccctgccccggttcatcctgctggagctcatggcggggggagacctcaagtccttcctccgagagacccgccctcgcccgagccagccctcctccctggccatgctggaccttctgcacgtggctcgggacattgcctgtggctgtcagtatttggaggaaaaccacttcatccaccgagacattgctgccagaaactgcctcttgacctgtccaggccctggaagagtggccaagattggagacttcgggatggcccgagacatctacagggcgagctactatagaaagggaggctgtgccatgctgccagttaagtggatgcccccagaggccttcatggaaggaatattcacttctaaaacagacacatggtcctttggagtgctgctatgggaaatcttttctcttggatatatgccataccccagcaaaagcaaccaggaagttctggagtttgtcaccagtggaggccggatggacccacccaagaactgccctgggcctgtataccggataatgactcagtgctggcaacatcagcctgaagacaggcccaactttgccatcattttggagaggattgaatactgcacccaggacccggatgtaatcaacaccgctttgccgatagaatatggtccacttgtggaagaggaagagaaagtgcctgtgaggcccaaggaccctgagggggttcctcctctcctggtctctcaacaggcaaaacgggaggaggagcgcagcccagctgccccaccacctctgcctaccacctcctctggcaaggctgcaaagaaacccacagctgcagaggtctctgttcgagtccctagagggccggccgtggaagggggacacgtgaatatggcattctctcagtccaaccctccttcggagttgcacaaggtccacggatccagaaacaagcccaccagcttgtggaacccaacgtacggctcctggtttacagagaaacccaccaaaaagaataatcctatagcaaagaaggagccacacgacaggggtaacctggggctggagggaagctgtactgtcccacctaacgttgcaactgggagacttccgggggcctcactgctcctagagccctcttcgctgactgccaatatgaaggaggtacctctgttcaggctacgtcacttcccttgtgggaatgtcaattacggctaccagcaacagggcttgcccttagaagccgctactgcccctggagctggtcattacgaggataccattctgaaaagcaagaatagcatgaaccagcctgggccctga

SEQ ID NO: 13 - protein, 1129 aa, Homo sapiens [sequence omitted]

SEQ ID NO: 14 - DNA, 3926 bp, Homo sapiens
  source 1..3926: mol_type = unassigned DNA
ggcggcgcggcgcggcgctcgcggctgctgcctgggagggaggccgggcaggcggctgagcggcgcggctctcaacgtgacggggaagtggttcgggcggccgcggcttactaccccagggcgaacggacggacgacggaggcgggagccggtagccgagccgggcgacctagagaacgagcgggtcaggctcagcgtcggccactctgtcggtccgctgaatgaagtgcccgcccctctgagcccggagcccggcgctttccccgcaagatggacggtttcgccggcagtctcgatgatagtatttctgctgcaagtacttctgatgttcaagatcgcctgtcagctcttgagtcacgagttcagcaacaagaagatgaaatcactgtgctaaaggcggctttggctgatgttttgaggcgtcttgcaatctctgaagatcatgtggcctcagtgaaaaaatcagtctcaagtaaaggccaaccaagccctcgagcagttattcccatgtcctgtataaccaatggaagtggtgcaaacagaaaaccaagtcataccagtgctgtctcaattgcaggaaaagaaactctttcatctgctgctaaaagtggtacagaaaaaaagaaagaaaaaccacaaggacagagagaaaaaaaagaggaatctcattctaatgatcaaagtccacaaattcgagcatcaccttctccccagccctcttcacaacctctccaaatacacagacaaactccagaaagcaagaatgctactcccaccaaaagcataaaacgaccatcaccagctgaaaagtcacataattcttgggaaaattcagatgatagccgtaataaattgtcgaaaataccttcaacacccaaattaataccaaaagttaccaaaactgcagacaagcataaagatgtcatcatcaaccaagaaggagaatatattaaaatgtttatgcgcggtcggccaattaccatgttcattccttccgatgttgacaactatgatgacatcagaacggaactgcctcctgagaagctcaaactggagtgggcatatggttatcgaggaaaggactgtagagctaatgtttaccttcttccgaccggggaaatagtttatttcattgcatcagtagtagtactatttaattatgaggagagaactcagcgacactacctgggccatacagactgtgtgaaatgccttgctatacatcctgacaaaattaggattgcaactggacagatagctggcgtggataaagatggaaggcctctacaaccccacgtcagagtgtgggattctgttactctatccacactgcagattattggacttggcacttttgagcgtggagtaggatgcctggatttttcaaaagcagattcaggtgttcatttatgtgttattgatgactccaatgagcatatgcttactgtatgggactggcagaagaaagcaaaaggagcagaaataaagacaacaaatgaagttgttttggctgtggagtttcacccaacagatgcaaataccataattacatgcggtaaatctcatattttcttctggacctggagcggcaattcactaacaagaaaacagggaatttttgggaaatatgaaaagccaaaatttgtgcagtgtttagcattcttggggaatggagatgttcttactggagactcaggtggagtcatgcttatatggagcaaaactactgtagagcccacacctgggaaaggacctaaagtgtaccgccggaagcaccaggagctgcaagccatgcagatggagctgcagagccctgagtacaagctgagcaagctccgcacctcgaccatcatgaccgactacaaccccaactactgctttgctggcaagacctcctccatcagtgacctgaaggaggtgccgcggaaaaacatcaccctcattcggggtctgggccatggagcctttggggaggtgtatgaaggccaggtgtccggaatgcccaacgacccaagccccctgcaagtggctgtgaagacgctgcctgaagtgtgctctgaacaggacgaactggatttcctcatggaagccctgatcatcagcaaattcaaccaccagaacattgttcgctgcattggggtgagcctgcaatccctgccccggttcatcctgctggagctcatggcggggggagacctcaagtccttcctccgagagacccgccctcgcccgagccagccctcctccctggccatgctggaccttctgcacgtggctcgggacattgcctgtggctgtcagtatttggaggaaaaccacttcatccaccgagacattgctgccagaaactgcctcttgacctgtccaggccctggaagagtggccaagattggagacttcgggatggcccgagacatctacagggcgagctactatagaaagggaggctgtgccatgctgccagttaagtggatgcccccagaggccttcatggaaggaatattcacttctaaaacagacacatggtcctttggagtgctgctatgggaaatcttttctcttggatatatgccataccccagcaaaagcaaccaggaagttctggagtttgtcaccagtggaggccggatggacccacccaagaactgccctgggcctgtataccggataatgactcagtgctggcaacatcagcctgaagacaggcccaactttgccatcattttggagaggattgaatactgcacccaggacccggatgtaatcaacaccgctttgccgatagaatatggtccacttgtggaagaggaagagaaagtgcctgtgaggcccaaggaccctgagggggttcctcctctcctggtctctcaacaggcaaaacgggaggaggagcgcagcccagctgccccaccacctctgcctaccacctcctctggcaaggctgcaaagaaacccacagctgcagaggtctctgttcgagtccctagagggccggccgtggaagggggacacgtgaatatggcattctctcagtccaaccctccttcggagttgcacagggtccacggatccagaaacaagcccaccagcttgtggaacccaacgtacggctcctggtttacagagaaacccaccaaaaagaataatcctatagcaaagaaggagccacacgagaggggtaacctggggctggagggaagctgtactgtcccacctaacgttgcaactgggagacttccgggggcctcactgctcctagagccctcttcgctgactgccaatatgaaggaggtacctctgttcaggctacgtcacttcccttgtgggaatgtcaattacggctaccagcaacagggcttgcccttagaagccgctactgcccctggagctggtcattacgaggataccattctgaaaagcaagaatagcatgaaccagcctgggccctgagctcggtcacacactcacttctcttccttgggatccctaagaccgtggaggagagagaggcaatcaatggctccttcacaaaccagagaccaaatgtcacgttttgttttgtgccaacctattttgaagtaccaccaaaaaagctgtattttgaaaatgctttagaaaggttttgagcatgggttcatcctattctttcgaaagaagaaaatatcataaaaatgagtgataaatacaaggcccagatgtggttgcataaggtttttatgcatgtttgttgtatacttccttatgcttcttttaaattgtgtgtgctctgcttcaatgtagtcagaattagctgcttctatgtttcatagttggggtcatagatgtttccttgccttgttgatgtggacatgagccatttgaggggagagggaacggaaataaaggagttatttgtaatgaaaaaaaaaaaaaaaaaaaaaaaaaaa

SEQ ID NO: 15 - protein, 1059 aa, Homo sapiens [sequence omitted]

SEQ ID NO: 16 - protein, 10 aa, Homo sapiens
SLAMLDLLHV

SEQ ID NO: 17 - protein, 680 aa, Homo sapiens; identical to SEQ ID NO: 11

SEQ ID NO: 18 - protein, 9 aa, Homo sapiens
VLLWEIFSL

SEQ ID NO: 19 - protein, 9 aa, Homo sapiens
FLMEALIIS

SEQ ID NO: 20 - protein, 9 aa, Homo sapiens
KTDTWSFGV

SEQ ID NO: 21 - protein, 9 aa, Homo sapiens
GMARDIYRA

SEQ ID NO: 22 - protein, 10 aa, Homo sapiens
FLMEALIISK

SEQ ID NO: 23 - protein, 10 aa, Homo sapiens
SLPRFILLEL

SEQ ID NO: 24 - protein, 10 aa, Homo sapiens
LLLEPSSLTA

SEQ ID NO: 25 - protein, 10 aa, Homo sapiens
GVLLWEIFSL

SEQ ID NO: 26 - protein, 9 aa, Homo sapiens
KPTKKNNPI

SEQ ID NO: 27 - protein, 9 aa, Homo sapiens
RPSQPSSLA

SEQ ID NO: 28 - protein, 9 aa, Homo sapiens
LPRFILLEL

SEQ ID NO: 29 - protein, 9 aa, Homo sapiens
RPRPSQPSS

SEQ ID NO: 30 - protein, 10 aa, Homo sapiens
RPSQPSSLAM

SEQ ID NO: 31 - protein, 10 aa, Homo sapiens
YPSKSNQEVL

SEQ ID NO: 32 - protein, 10 aa, Homo sapiens
LPRFILLELM

SEQ ID NO: 33 - protein, 10 aa, Homo sapiens
SPLQVAVKTL

SEQ ID NO: 34 - protein, 9 aa, Homo sapiens
YYRKGGCAM

SEQ ID NO: 35 - protein, 9 aa, Homo sapiens
VYEGQVSGM

SEQ ID NO: 36 - protein, 9 aa, Homo sapiens
YRKGGCAML

SEQ ID NO: 37 - protein, 9 aa, Homo sapiens
VYRRKHQEL

SEQ ID NO: 38 - protein, 9 aa, Homo sapiens
KWMPPEAFM

SEQ ID NO: 39 - protein, 9 aa, Homo sapiens
VRVPRGPAV

SEQ ID NO: 40 - protein, 9 aa, Homo sapiens
GRLPGASLL

SEQ ID NO: 41 - protein, 10 aa, Homo sapiens
YYRKGGCAML

SEQ ID NO: 42 - protein, 10 aa, Homo sapiens
SYYRKGGCAM

SEQ ID NO: 43 - protein, 10 aa, Homo sapiens
ERSPAAPPPL

SEQ ID NO: 44 - protein, 10 aa, Homo sapiens
RRKHQELQAM

SEQ ID NO: 45 - protein, 11 aa, Homo sapiens
ERSAPAAPPPL

SEQ ID NO: 46 - protein, 10 aa, Homo sapiens
GRLPGASLLL

SEQ ID NO: 47 - protein, 10 aa, Homo sapiens
SFGVLLWEIF

SEQ ID NO: 48 - protein, 36 aa, synthetic construct
  REGION 1..36: note = Description of Artificial Sequence: Synthetic polypeptide
VYRRKHQELQAMQMELQSPEYKLSKLRTSTIMTDYN

SEQ ID NO: 49 - protein, 36 aa, synthetic construct
  REGION 1..36: note = Description of Artificial Sequence: Synthetic polypeptide
KLRTSTIMTDYNPNYCFAGKTSSISDLKEVPRKNIT

SEQ ID NO: 50 - protein, 36 aa, synthetic construct
  REGION 1..36: note = Description of Artificial Sequence: Synthetic polypeptide
SDLKEVPRKNITLIRGLGHGAFGEVYEGQVSGMPND

SEQ ID NO: 51 - protein, 36 aa, synthetic construct
  REGION 1..36: note = Description of Artificial Sequence: Synthetic polypeptide
VYEGQVSGMPNDPSPLQVAVKTLPEVCSEQDELDFL

SEQ ID NO: 52 - protein, 36 aa, synthetic construct
  REGION 1..36: note = Description of Artificial Sequence: Synthetic polypeptide
EVCSEQDELDFLMEALIISKFNHQNIVRCIGVSLQS

SEQ ID NO: 53 - protein, 36 aa, synthetic construct
  REGION 1..36: note = Description of Artificial Sequence: Synthetic polypeptide
NIVRCIGVSLQSLPRFILLELMAGGDLKSFLRETRP

SEQ ID NO: 54 - protein, 36 aa, synthetic construct
  REGION 1..36: note = Description of Artificial Sequence: Synthetic polypeptide
GDLKSFLRETRPRPSQPSSLAMLDLLHVARDIACGC

SEQ ID NO: 55 - protein, 36 aa, synthetic construct
  REGION 1..36: note = Description of Artificial Sequence: Synthetic polypeptide
LLHVARDIACGCQYLEENHFIHRDIAARNCLLTCPG

SEQ ID NO: 56 - protein, 36 aa, synthetic construct
  REGION 1..36: note = Description of Artificial Sequence: Synthetic polypeptide
IAARNCLLTCPGPGRVAKIGDFGMARDIYRASYYRK

SEQ ID NO: 57 - protein, 36 aa, synthetic construct
  REGION 1..36: note = Description of Artificial Sequence: Synthetic polypeptide
ARDIYRASYYRKGGCAMLPVKWMPPEAFMEGIFTSK

SEQ ID NO: 58 - protein, 36 aa, synthetic construct
  REGION 1..36: note = Description of Artificial Sequence: Synthetic polypeptide
PEAFMEGIFTSKTDTWSFGVLLWEIFSLGYMPYPSK

SEQ ID NO: 59 - protein, 36 aa, synthetic construct
  REGION 1..36: note = Description of Artificial Sequence: Synthetic polypeptide
IFSLGYMPYPSKSNQEVLEFVTSGGRMDPPKNCPGP

SEQ ID NO: 60 - protein, 36 aa, synthetic construct
  REGION 1..36: note = Description of Artificial Sequence: Synthetic polypeptide
GRMDPPKNCPGPVYRIMTQCWQHQPEDRPNFAIILE

SEQ ID NO: 61 - protein, 36 aa, synthetic construct
  REGION 1..36: note = Description of Artificial Sequence: Synthetic polypeptide
PEDRPNFAIILERIEYCTQDPDVINTALPIEYGPLV

SEQ ID NO: 62 - protein, 36 aa, synthetic construct
  REGION 1..36: note = Description of Artificial Sequence: Synthetic polypeptide
NTALPIEYGPLVEEEEKVPVRPKDPEGVPPLLVSQQ

SEQ ID NO: 63 - protein, 36 aa, synthetic construct
  REGION 1..36: note = Description of Artificial Sequence: Synthetic polypeptide
PEGVPPLLVSQQAKREEERSPAAPPPLPTTSSGKAA

SEQ ID NO: 64 - protein, 36 aa, synthetic construct
  REGION 1..36: note = Description of Artificial Sequence: Synthetic polypeptide
PPLPTTSSGKAAKKPTAAEISVRVPRGPAVEGGHVN

SEQ ID NO: 65 - protein, 36 aa, synthetic construct
  REGION 1..36: note = Description of Artificial Sequence: Synthetic polypeptide
PRGPAVEGGHVNMAFSQSNPPSELHKVHGSRNKPTS

SEQ ID NO: 66 - protein, 36 aa, synthetic construct
  REGION 1..36: note = Description of Artificial Sequence: Synthetic polypeptide
HKVHGSRNKPTSLWNPTYGSWFTEKPTKKNNPIAKK

SEQ ID NO: 67 - protein, 36 aa, synthetic construct
  REGION 1..36: note = Description of Artificial Sequence: Synthetic polypeptide
KPTKKNNPIAKKEPHDRGNLGLEGSCTVPPNVATGR

SEQ ID NO: 68 - protein, 36 aa, synthetic construct
  REGION 1..36: note = Description of Artificial Sequence: Synthetic polypeptide
SCTVPPNVATGRLPGASLLLEPSSLTANMKEVPLFR

SEQ ID NO: 69 - protein, 36 aa, synthetic construct
  REGION 1..36: note = Description of Artificial Sequence: Synthetic polypeptide
LTANMKEVPLFRLRHFPCGNVNYGYQQQGLPLEAAT

SEQ ID NO: 70 - protein, 36 aa, synthetic construct
  REGION 1..36: note = Description of Artificial Sequence: Synthetic polypeptide
GYQQQGLPLEAATAPGAGHYEDTILKSKNSMNQPGP

SEQ ID NO: 71 - protein, 9 aa, Homo sapiens
PGPGRVAKI

SEQ ID NO: 72 - protein, 19 aa, Homo sapiens
PGPGRVAKIGDFGMARDIY

SEQ ID NO: 73 - protein, 19 aa, Homo sapiens
CGNVNYGYQQQGLPLEAAT

SEQ ID NO: 74 - protein, 8 aa, Homo sapiens
PRKNITLI

SEQ ID NO: 75 - protein, 70 aa, Homo sapiens
WVRRGRQDFGRPCPERPQLLPPGPLQCLRTLRSRGAGESKDAANLRSAGAGIHAQKFSRQTVRSLPAAER

SEQ ID NO: 76 - protein, 45 aa, Homo sapiens
LEGAQDGSLRPRFPPRPGRRAWRSQKERKRRPGQRAAAGSRRSQP

SEQ ID NO: 77 - protein, 63 aa, Homo sapiens
KLQRLEAAPRGDRPQLRLRGAGEDGTQLPPPFNHSSSSVPSAASYRRGRGTRRGEREAQGPSQ

SEQ ID NO: 78 - protein, 4 aa, Homo sapiens
AQCA

SEQ ID NO: 79 - protein, 14 aa, Homo sapiens
VSLDSPLSFQVCFI

SEQ ID NO: 80 - protein, 46 aa, Homo sapiens
TPARLRAVGGKQETCAHAQSSGDQVEGAAGYQGLFRASSHLGESEG

SEQ ID NO: 81 - protein, 7 aa, Homo sapiens
GWARRAV

SEQ ID NO: 82 - protein, 1626 aa, Homo sapiens; identical to SEQ ID NO: 6

SEQ ID NO: 83 - protein, 40 aa, Homo sapiens
ARSHTHFSSLGSLRPWRRERQWLLHKPETKCHVLFCANLF

SEQ ID NO: 84 - protein, 8 aa, Homo sapiens
STTKKAVF

SEQ ID NO: 85 - protein, 24 aa, Homo sapiens
KCFRKVLSMGSSYSFERRKYHKNE

SEQ ID NO: 86 - protein, 8 aa, Homo sapiens
IQGPDVVA

SEQ ID NO: 87 - protein, 26 aa, Homo sapiens
GFYACLLYTSLCFFQIVCALLQCSQN

SEQ ID NO: 88 - protein, 16 aa, Homo sapiens
LLLCFIVGVIDVSLPC

SEQ ID NO: 89 - protein, 20 aa, Homo sapiens
CGHEPFEGRGNGNKGVICND